European Patent Specification EP 3 618 928 B1, published January 18, 2023. Title: ANTI-SORTILIN ANTIBODIES AND METHODS OF USE THEREOF. Applicant: Alector LLC. Application Not Yet Assigned. The sequence listing filed with the application follows.

SEQUENCE LISTING (146 sequences)

SEQ ID NO: 1 - protein, 10 aa, Artificial Sequence
  Synthetic Construct
YSISSGYYWG

SEQ ID NO: 2 - protein, 16 aa, Artificial Sequence
  Synthetic Construct
TIYHSGSTYYNPSLKS

SEQ ID NO: 3 - protein, 16 aa, Artificial Sequence
  Synthetic Construct
TIYHSGSTYYNPSLES

SEQ ID NO: 4 - protein, 16 aa, Artificial Sequence
  Synthetic Construct
  VARIANT 15: Xaa = Lys or Glu
TIYHSGSTYYNPSLXS

SEQ ID NO: 5 - protein, 15 aa, Artificial Sequence
  Synthetic Construct
ARQGSIQQGYYGMDV

SEQ ID NO: 6 - protein, 15 aa, Artificial Sequence
  Synthetic Construct
ARQGSIKQGYYGMDV

SEQ ID NO: 7 - protein, 15 aa, Artificial Sequence
  Synthetic Construct
  VARIANT 7: Xaa = Gln or Lys
ARQGSIXQGYYGMDV

SEQ ID NO: 8 - protein, 16 aa, Artificial Sequence
  Synthetic Construct
RSSQSLLRSNGYNYLD

SEQ ID NO: 9 - protein, 16 aa, Artificial Sequence
  Synthetic Construct
RSSQSLLRSTGYNYLD

SEQ ID NO: 10 - protein, 16 aa, Artificial Sequence
  Synthetic Construct
RSSQSLLRSSGYNYLD

SEQ ID NO: 11 - protein, 16 aa, Artificial Sequence
  Synthetic Construct
RSSQSLLRSGGYNYLD

SEQ ID NO: 12 - protein, 16 aa, Artificial Sequence
  Synthetic Construct
RSSQSLLRSRGYNYLD

SEQ ID NO: 13 - protein, 16 aa, Artificial Sequence
  Synthetic Construct
RSSQSLLRSDGYNYLD

SEQ ID NO: 14 - protein, 16 aa, Artificial Sequence
  Synthetic Construct
RSSQSLLRSHGYNYLD

SEQ ID NO: 15 - protein, 16 aa, Artificial Sequence
  Synthetic Construct
RSSQSLLRSKGYNYLD

SEQ ID NO: 16 - protein, 16 aa, Artificial Sequence
  Synthetic Construct
RSSQSLLRSQGYNYLD

SEQ ID NO: 17 - protein, 16 aa, Artificial Sequence
  Synthetic Construct
RSSQSLLRSYGYNYLD

SEQ ID NO: 18 - protein, 16 aa, Artificial Sequence
  Synthetic Construct
RSSQSLLRSEGYNYLD

SEQ ID NO: 19 - protein, 16 aa, Artificial Sequence
  Synthetic Construct
RSSQSLLRSWGYNYLD

SEQ ID NO: 20 - protein, 16 aa, Artificial Sequence
  Synthetic Construct
RSSQSLLRSFGYNYLD

SEQ ID NO: 21 - protein, 16 aa, Artificial Sequence
  Synthetic Construct
RSSQSLLRSIGYNYLD

SEQ ID NO: 22 - protein, 16 aa, Artificial Sequence
  Synthetic Construct
RSSQSLLRSVGYNYLD

SEQ ID NO: 23 - protein, 16 aa, Artificial Sequence
  Synthetic Construct
RSSQSLLRSAGYNYLD

SEQ ID NO: 24 - protein, 16 aa, Artificial Sequence
  Synthetic Construct
RSSQSLLRSMGYNYLD

SEQ ID NO: 25 - protein, 16 aa, Artificial Sequence
  Synthetic Construct
RSSQSLLRSLGYNYLD

SEQ ID NO: 26 - protein, 16 aa, Artificial Sequence
  Synthetic Construct
RSSQSLLHSNGYNYLD

SEQ ID NO: 27 - protein, 16 aa, Artificial Sequence
  Synthetic Construct
RSSQGLLRSNGYNYLD

SEQ ID NO: 28 - protein, 16 aa, Artificial Sequence
  Synthetic Construct
  VARIANT 5: Xaa = Ser or Gly
  VARIANT 8: Xaa = Arg or His
  VARIANT 10: Xaa = Asn, Thr, Ser, Gly, Arg, Asp, His, Lys, Gln, Tyr, Glu, Trp, Phe, Ile, Val, Ala, Met, or Leu
RSSQXLLXSXGYNYLD

SEQ ID NO: 29 - protein, 7 aa, Artificial Sequence
  Synthetic Construct
LGSNRAS

SEQ ID NO: 30 - protein, 7 aa, Artificial Sequence
  Synthetic Construct
LGSNRVS

SEQ ID NO: 31 - protein, 7 aa, Artificial Sequence
  Synthetic Construct
  VARIANT 6: Xaa = Ala or Val
LGSNRXS

SEQ ID NO: 32 - protein, 9 aa, Artificial Sequence
  Synthetic Construct
MQQQEAPLT

SEQ ID NO: 33 - protein, 9 aa, Artificial Sequence
  Synthetic Construct
MQQQETPLT

SEQ ID NO: 34 - protein, 9 aa, Artificial Sequence
  Synthetic Construct
  VARIANT 6: Xaa = Ala or Thr
MQQQEXPLT

SEQ ID NO: 35 - protein, 26 aa, Artificial Sequence
  Synthetic Construct
QVQLQESGPGLVKPSETLSLTCAVSG

SEQ ID NO: 36 - protein, 14 aa, Artificial Sequence
  Synthetic Construct
WIRQPPGKGLEWIG

SEQ ID NO: 37 - protein, 30 aa, Artificial Sequence
  Synthetic Construct
QVTISVDTSKNQFSLELSSVTAADTAVYYC

SEQ ID NO: 38 - protein, 30 aa, Artificial Sequence
  Synthetic Construct
RVTISVDTSKNQFSLKLSSVTAADTAVYYC

SEQ ID NO: 39 - protein, 30 aa, Artificial Sequence
  Synthetic Construct
  VARIANT 1: Xaa = Gln or Arg
  VARIANT 16: Xaa = Glu or Lys
XVTISVDTSKNQFSLXLSSVTAADTAVYYC

SEQ ID NO: 40 - protein, 11 aa, Artificial Sequence
  Synthetic Construct
WGQGTTVTVSS

SEQ ID NO: 41 - protein, 23 aa, Artificial Sequence
  Synthetic Construct
DIVMTQSPLSLPVTPGEPASISC

SEQ ID NO: 42 - protein, 23 aa, Artificial Sequence
  Synthetic Construct
DIVMTQSPLSLPVTPGGPASISC

SEQ ID NO: 43 - protein, 23 aa, Artificial Sequence
  Synthetic Construct
DIVMTQSPLSLPVTPGESASISC

SEQ ID NO: 44 - protein, 23 aa, Artificial Sequence
  Synthetic Construct
  VARIANT 17: Xaa = Glu or Gly
  VARIANT 18: Xaa = Pro or Ser
DIVMTQSPLSLPVTPGXXASISC

SEQ ID NO: 45 - protein, 15 aa, Artificial Sequence
  Synthetic Construct
WYLQKPGQSPQLLIY

SEQ ID NO: 46 - protein, 15 aa, Artificial Sequence
  Synthetic Construct
WYLQKPGQPPQLLIY

SEQ ID NO: 47 - protein, 15 aa, Artificial Sequence
  Synthetic Construct
  VARIANT 9: Xaa = Ser or Pro
WYLQKPGQXPQLLIY

SEQ ID NO: 48 - protein, 32 aa, Artificial Sequence
  Synthetic Construct
GVPDRFSGSGSGTDFTLKISRAEAEDVGVYYC

SEQ ID NO: 49 - protein, 32 aa, Artificial Sequence
  Synthetic Construct
GVPDRFSGSGSGTDFTLKISRVEAEDVGVYYC

SEQ ID NO: 50 - protein, 32 aa, Artificial Sequence
  Synthetic Construct
GVPDRFSGSGSGTDFTLKISRVEAEDVGAYYC

SEQ ID NO: 51 - protein, 32 aa, Artificial Sequence
  Synthetic Construct
GVPDRLSGSGSGTDFTLKISRVEAEDVGVYYC

SEQ ID NO: 52 - protein, 32 aa, Artificial Sequence
  Synthetic Construct
  VARIANT 6: Xaa = Phe or Leu
  VARIANT 22: Xaa = Ala or Val
  VARIANT 29: Xaa = Val or Ala
GVPDRXSGSGSGTDFTLKISRXEAEDVGXYYC

SEQ ID NO: 53 - protein, 10 aa, Artificial Sequence
  Synthetic Construct
FGGGTKVEIK

SEQ ID NO: 54 - protein, 122 aa, Artificial Sequence
  Synthetic Construct
QVQLQESGPGLVKPSETLSLTCAVSGYSISSGYYWGWIRQPPGKGLEWIGTIYHSGSTYYNPSLKSQVTISVDTSKNQFSLELSSVTAADTAVYYCARQGSIQQGYYGMDVWGQGTTVTVSS

SEQ ID NO: 55 - protein, 122 aa, Artificial Sequence
  Synthetic Construct
QVQLQESGPGLVKPSETLSLTCAVSGYSISSGYYWGWIRQPPGKGLEWIGTIYHSGSTYYNPSLESRVTISVDTSKNQFSLKLSSVTAADTAVYYCARQGSIQQGYYGMDVWGQGTTVTVSS

SEQ ID NO: 56 - protein, 122 aa, Artificial Sequence
  Synthetic Construct
QVQLQESGPGLVKPSETLSLTCAVSGYSISSGYYWGWIRQPPGKGLEWIGTIYHSGSTYYNPSLKSRVTISVDTSKNQFSLKLSSVTAADTAVYYCARQGSIKQGYYGMDVWGQGTTVTVSS

SEQ ID NO: 57 - protein, 112 aa, Artificial Sequence
  Synthetic Construct
DIVMTQSPLSLPVTPGEPASISCRSSQSLLRSNGYNYLDWYLQKPGQSPQLLIYLGSNRASGVPDRFSGSGSGTDFTLKISRAEAEDVGVYYCMQQQEAPLTFGGGTKVEIK

SEQ ID NO: 58 - protein, 112 aa, Artificial Sequence
  Synthetic Construct
DIVMTQSPLSLPVTPGEPASISCRSSQSLLRSNGYNYLDWYLQKPGQSPQLLIYLGSNRASGVPDRFSGSGSGTDFTLKISRVEAEDVGVYYCMQQQEAPLTFGGGTKVEIK

SEQ ID NO: 59 - protein, 112 aa, Artificial Sequence
  Synthetic Construct
DIVMTQSPLSLPVTPGEPASISCRSSQSLLRSNGYNYLDWYLQKPGQPPQLLIYLGSNRVSGVPDRFSGSGSGTDFTLKISRVEAEDVGVYYCMQQQETPLTFGGGTKVEIK

SEQ ID NO: 60 - protein, 112 aa, Artificial Sequence
  Synthetic Construct
DIVMTQSPLSLPVTPGEPASISCRSSQSLLRSTGYNYLDWYLQKPGQSPQLLIYLGSNRASGVPDRFSGSGSGTDFTLKISRAEAEDVGVYYCMQQQEAPLTFGGGTKVEIK

SEQ ID NO: 61 - protein, 112 aa, Artificial Sequence
  Synthetic Construct
DIVMTQSPLSLPVTPGEPASISCRSSQSLLRSSGYNYLDWYLQKPGQSPQLLIYLGSNRASGVPDRFSGSGSGTDFTLKISRAEAEDVGVYYCMQQQEAPLTFGGGTKVEIK

SEQ ID NO: 62 - protein, 112 aa, Artificial Sequence
  Synthetic Construct
DIVMTQSPLSLPVTPGEPASISCRSSQSLLRSGGYNYLDWYLQKPGQSPQLLIYLGSNRASGVPDRFSGSGSGTDFTLKISRAEAEDVGVYYCMQQQEAPLTFGGGTKVEIK

SEQ ID NO: 63 - protein, 112 aa, Artificial Sequence
  Synthetic Construct
DIVMTQSPLSLPVTPGEPASISCRSSQSLLRSRGYNYLDWYLQKPGQSPQLLIYLGSNRASGVPDRFSGSGSGTDFTLKISRAEAEDVGVYYCMQQQEAPLTFGGGTKVEIK

SEQ ID NO: 64 - protein, 112 aa, Artificial Sequence
  Synthetic Construct
DIVMTQSPLSLPVTPGEPASISCRSSQSLLRSDGYNYLDWYLQKPGQSPQLLIYLGSNRASGVPDRFSGSGSGTDFTLKISRAEAEDVGVYYCMQQQEAPLTFGGGTKVEIK

SEQ ID NO: 65 - protein, 112 aa, Artificial Sequence
  Synthetic Construct
DIVMTQSPLSLPVTPGEPASISCRSSQSLLRSHGYNYLDWYLQKPGQSPQLLIYLGSNRASGVPDRFSGSGSGTDFTLKISRAEAEDVGVYYCMQQQEAPLTFGGGTKVEIK

SEQ ID NO: 66 - protein, 112 aa, Artificial Sequence
  Synthetic Construct
DIVMTQSPLSLPVTPGEPASISCRSSQSLLRSKGYNYLDWYLQKPGQSPQLLIYLGSNRASGVPDRFSGSGSGTDFTLKISRAEAEDVGVYYCMQQQEAPLTFGGGTKVEIK

SEQ ID NO: 67 - protein, 112 aa, Artificial Sequence
  Synthetic Construct
DIVMTQSPLSLPVTPGEPASISCRSSQSLLRSQGYNYLDWYLQKPGQSPQLLIYLGSNRASGVPDRFSGSGSGTDFTLKISRAEAEDVGVYYCMQQQEAPLTFGGGTKVEIK

SEQ ID NO: 68 - protein, 112 aa, Artificial Sequence
  Synthetic Construct
DIVMTQSPLSLPVTPGEPASISCRSSQSLLRSYGYNYLDWYLQKPGQSPQLLIYLGSNRASGVPDRFSGSGSGTDFTLKISRAEAEDVGVYYCMQQQEAPLTFGGGTKVEIK

SEQ ID NO: 69 - protein, 112 aa, Artificial Sequence
  Synthetic Construct
DIVMTQSPLSLPVTPGEPASISCRSSQSLLRSEGYNYLDWYLQKPGQSPQLLIYLGSNRASGVPDRFSGSGSGTDFTLKISRAEAEDVGVYYCMQQQEAPLTFGGGTKVEIK

SEQ ID NO: 70 - protein, 112 aa, Artificial Sequence
  Synthetic Construct
DIVMTQSPLSLPVTPGEPASISCRSSQSLLRSWGYNYLDWYLQKPGQSPQLLIYLGSNRASGVPDRFSGSGSGTDFTLKISRAEAEDVGVYYCMQQQEAPLTFGGGTKVEIK

SEQ ID NO: 71 - protein, 112 aa, Artificial Sequence
  Synthetic Construct
DIVMTQSPLSLPVTPGEPASISCRSSQSLLRSFGYNYLDWYLQKPGQSPQLLIYLGSNRASGVPDRFSGSGSGTDFTLKISRAEAEDVGVYYCMQQQEAPLTFGGGTKVEIK

SEQ ID NO: 72 - protein, 112 aa, Artificial Sequence
  Synthetic Construct
DIVMTQSPLSLPVTPGEPASISCRSSQSLLRSIGYNYLDWYLQKPGQSPQLLIYLGSNRASGVPDRFSGSGSGTDFTLKISRAEAEDVGVYYCMQQQEAPLTFGGGTKVEIK

SEQ ID NO: 73 - protein, 112 aa, Artificial Sequence
  Synthetic Construct
DIVMTQSPLSLPVTPGEPASISCRSSQSLLRSVGYNYLDWYLQKPGQSPQLLIYLGSNRASGVPDRFSGSGSGTDFTLKISRAEAEDVGVYYCMQQQEAPLTFGGGTKVEIK

SEQ ID NO: 74 - protein, 112 aa, Artificial Sequence
  Synthetic Construct
DIVMTQSPLSLPVTPGEPASISCRSSQSLLRSAGYNYLDWYLQKPGQSPQLLIYLGSNRASGVPDRFSGSGSGTDFTLKISRAEAEDVGVYYCMQQQEAPLTFGGGTKVEIK

SEQ ID NO: 75 - protein, 112 aa, Artificial Sequence
  Synthetic Construct
DIVMTQSPLSLPVTPGEPASISCRSSQSLLRSMGYNYLDWYLQKPGQSPQLLIYLGSNRASGVPDRFSGSGSGTDFTLKISRAEAEDVGVYYCMQQQEAPLTFGGGTKVEIK

SEQ ID NO: 76 - protein, 112 aa, Artificial Sequence
  Synthetic Construct
DIVMTQSPLSLPVTPGEPASISCRSSQSLLRSLGYNYLDWYLQKPGQSPQLLIYLGSNRASGVPDRFSGSGSGTDFTLKISRAEAEDVGVYYCMQQQEAPLTFGGGTKVEIK

SEQ ID NO: 77 - protein, 112 aa, Artificial Sequence
  Synthetic Construct
DIVMTQSPLSLPVTPGEPASISCRSSQSLLRSNGYNYLDWYLQKPGQSPQLLIYLGSNRASGVPDRFSGSGSGTDFTLKISRVEAEDVGAYYCMQQQEAPLTFGGGTKVEIK

SEQ ID NO: 78 - protein, 112 aa, Artificial Sequence
  Synthetic Construct
DIVMTQSPLSLPVTPGGPASISCRSSQSLLRSNGYNYLDWYLQKPGQSPQLLIYLGSNRASGVPDRLSGSGSGTDFTLKISRVEAEDVGVYYCMQQQETPLTFGGGTKVEIK

SEQ ID NO: 79 - protein, 112 aa, Artificial Sequence
  Synthetic Construct
DIVMTQSPLSLPVTPGEPASISCRSSQSLLHSNGYNYLDWYLQKPGQSPQLLIYLGSNRASGVPDRFSGSGSGTDFTLKISRVEAEDVGVYYCMQQQETPLTFGGGTKVEIK

SEQ ID NO: 80 - protein, 112 aa, Artificial Sequence
  Synthetic Construct
DIVMTQSPLSLPVTPGESASISCRSSQGLLRSNGYNYLDWYLQKPGQSPQLLIYLGSNRASGVPDRFSGSGSGTDFTLKISRVEAEDVGVYYCMQQQEAPLTFGGGTKVEIK

SEQ ID NO: 81 - protein, 831 aa, Homo sapiens
MERPWGAADGLSRWPHGLGLLLLLQLLPPSTLSQDRLDAPPPPAAPLPRWSGPIGVSWGLRAAAAGGAFPRGGRWRRSAPGEDEECGRVRDFVAKLANNTHQHVFDDLRGSVSLSWVGDSTGVILVLTTFHVPLVIMTFGQSKLYRSEDYGKNFKDITDLINNTFIRTEFGMAIGPENSGKVVLTAEVSGGSRGGRIFRSSDFAKNFVQTDLPFHPLTQMMYSPQNSDYLLALSTENGLWVSKNFGGKWEEIHKAVCLAKWGSDNTIFFTTYANGSCKADLGALELWRTSDLGKSFKTIGVKIYSFGLGGRFLFASVMADKDTTRRIHVSTDQGDTWSMAQLPSVGQEQFYSILAANDDMVFMHVDEPGDTGFGTIFTSDDRGIVYSKSLDRHLYTTTGGETDFTNVTSLRGVYITSVLSEDNSIQTMITFDQGGRWTHLRKPENSECDATAKNKNECSLHIHASYSISQKLNVPMAPLSEPNAVGIVIAHGSVGDAISVMVPDVYISDDGGYSWTKMLEGPHYYTILDSGGIIVAIEHSSRPINVIKFSTDEGQCWQTYTFTRDPIYFTGLASEPGARSMNISIWGFTESFLTSQWVSYTIDFKDILERNCEEKDYTIWLAHSTDPEDYEDGCILGYKEQFLRLRKSSVCQNGRDYVVTKQPSICLCSLEDFLCDFGYYRPENDSKCVEQPELKGHDLEFCLYGREEHLTTNGYRKIPGDKCQGGVNPVREVKDLKKKCTSNFLSPEKQNSKSNSVPIILAIVGLMLVTVVAGVLIVKKYVCGGRFLVHRYSVLQQHAEANGVDGVDALDTASHTNKSGYHDDSDEDLLE

SEQ ID NO: 82 - protein, 825 aa, Mus musculus
MERPRGAADGLLRWPLGLLLLLQLLPPAAVGQDRLDAPPPPAPPLLRWAGPVGVSWGLRAAAPGGPVPRAGRWRRGAPAEDQDCGRLPDFIAKLTNNTHQHVFDDLSGSVSLSWVGDSTGVILVLTTFQVPLVIVSFGQSKLYRSEDYGKNFKDITNLINNTFIRTEFGMAIGPENSGKVILTAEVSGGSRGGRVFRSSDFAKNFVQTDLPFHPLTQMMYSPQNSDYLLALSTENGLWVSKNFGEKWEEIHKAVCLAKWGPNNIIFFTTHVNGSCKADLGALELWRTSDLGKTFKTIGVKIYSFGLGGRFLFASVMADKDTTRRIHVSTDQGDTWSMAQLPSVGQEQFYSILAANEDMVFMHVDEPGDTGFGTIFTSDDRGIVYSKSLDRHLYTTTGGETDFTNVTSLRGVYITSTLSEDNSIQSMITFDQGGRWEHLRKPENSKCDATAKNKNECSLHIHASYSISQKLNVPMAPLSEPNAVGIVIAHGSVGDAISVMVPDVYISDDGGYSWAKMLEGPHYYTILDSGGIIVAIEHSNRPINVIKFSTDEGQCWQSYVFTQEPIYFTGLASEPGARSMNISIWGFTESFITRQWVSYTVDFKDILERNCEEDDYTTWLAHSTDPGDYKDGCILGYKEQFLRLRKSSVCQNGRDYVVAKQPSVCPCSLEDFLCDFGYFRPENASECVEQPELKGHELEFCLYGKEEHLTTNGYRKIPGDKCQGGMNPAREVKDLKKKCTSNFLNPTKQNSKSNSVPIILAIVGLMLVTVVAGVLIVKKYVCGGRFLVHRYSVLQQHAEADGVEALDSTSHAKSGYHDDSDEDLLE

SEQ ID NO: 83 - protein, 825 aa, Rattus norvegicus
MERPRGAADGLLRWPLGLLLLLQLLPPAAVGQDRLDAPPPPAPPLLRWAGPVGVSWGLRAAAPGGPVPRAGRWRRGAPAEDQDCGRLPDFIAKLTNNTHQHVFDDLSGSVSLSWVGDSTGVILVLTTFQVPLVIVSFGQSKLYRSEDYGKNFKDITNLINNTFIRTEFGMAIGPENSGKVILTAEVSGGSRGGRVFRSSDFAKNFVQTDLPFHPLTQMMYSPQNSDYLLALSTENGLWVSKNFGEKWEEIHKAVCLAKWGPNNIIFFTTHVNGSCKADLGALELWRTSDLGKTFKTIGVKIYSFGLGGRFLFASVMADKDTTRRIHVSTDQGDTWSMAQLPSVGQEQFYSILAANDDMVFMHVDEPGDTGFGTIFTSDDRGIVYSKSLDRHLYTTTGGETDFTNVTSLRGVYITSTLSEDNSIQSMITFDQGGRWEHLQKPENSKCDATAKNKNECSLHIHASYSISQKLNVPMAPLSEPNAVGIVIAHGSVGDAISVMVPDVYISDDGGYSWAKMLEGPHYYTILDSGGIIVAIEHSNRPINVIKFSTDEGQCWQSYVFSQEPVYFTGLASEPGARSMNISIWGFTESFLTRQWVSYTIDFKDILERNCEENDYTTWLAHSTDPGDYKDGCILGYKEQFLRLRKSSVCQNGRDYVVAKQPSICPCSLEDFLCDFGYFRPENASECVEQPELKGHELEFCLYGKEEHLTTNGYRKIPGDRCQGGMNPAREVKDLKKKCTSNFLNPKKQNSKSSSVPIILAIVGLMLVTVVAGVLIVKKYVCGGRFLVHRYSVLQQHAEADGVEALDTASHAKSGYHDDSDEDLLE

SEQ ID NO: 84 - protein, 8 aa, Artificial Sequence
  Synthetic Construct
  VARIANT 1: Xaa = Ser or Thr
  VARIANT 2: Xaa = Any Amino Acid
  VARIANT 3: Xaa = Asp or Asn
  VARIANT 4, 5, 6, 7: Xaa = Any Amino Acid
  VARIANT 8: Xaa = Trp, Phe, or Tyr
XXXXXXXX

SEQ ID NO: 85 - protein, 11 aa, Artificial Sequence
  Synthetic Construct
  VARIANT 1, 2: Xaa = Any Amino Acid
  VARIANT 3: Xaa = Ser or Thr
  VARIANT 4: Xaa = Any Amino Acid
  VARIANT 5: Xaa = Asp or Asn
  VARIANT 6, 8: Xaa = Any Amino Acid
  VARIANT 9: Xaa = Thr or Ser
  VARIANT 10: Xaa = Trp, Phe, or Tyr
  VARIANT 11: Xaa = Any Amino Acid
XXXXXXGXXXX

SEQ ID NO: 86 - protein, 8 aa, Artificial Sequence
  Synthetic Construct
SSDFAKNF

SEQ ID NO: 87 - protein, 6 aa, Artificial Sequence
  Synthetic Construct
NQFSLK

SEQ ID NO: 88 - protein, 23 aa, Artificial Sequence
  Synthetic Construct
QGYYGMDVWGQGTTVTVSSASTK

SEQ ID NO: 89 - protein, 49 aa, Artificial Sequence
  Synthetic Construct
DYFPEPVTVSWNSGALTSGVHTFPAVLQSSGLYSLSSVVTVPSSSLGTK

SEQ ID NO: 90 - protein, 7 aa, Artificial Sequence
  Synthetic Construct
DTLMISR

SEQ ID NO: 91 - protein, 33 aa, Artificial Sequence
  Synthetic Construct
TPEVTCVVVDVSQEDPEVQFNWYVDGVEVHNAK

SEQ ID NO: 92 - protein, 16 aa, Artificial Sequence
  Synthetic Construct
VVSVLTVLHQDWLNGK

SEQ ID NO: 93 - protein, 16 aa, Artificial Sequence
  Synthetic Construct
EPQVYTLPPSQEEMTK

SEQ ID NO: 94 - protein, 10 aa, Artificial Sequence
  Synthetic Construct
NQVSLTCLVK

SEQ ID NO: 95 - protein, 22 aa, Artificial Sequence
  Synthetic Construct
GFYPSDIAVEWESNGQPENNYK

SEQ ID NO: 96 - protein, 23 aa, Artificial Sequence
  Synthetic Construct
WQEGNVFSCSVMHEALHNHYTQK

SEQ ID NO: 97 - protein, 24 aa, Artificial Sequence
  Synthetic Construct
DIVMTQSPLSLPVTPGEPASISCR

SEQ ID NO: 98 - protein, 7 aa, Artificial Sequence
  Synthetic Construct
SSQSLLR

SEQ ID NO: 99 - protein, 28 aa, Artificial Sequence
  Synthetic Construct
SNGYNYLDWYLQKPGQSPQLLIYLGSNR

SEQ ID NO: 100 - protein, 26 aa, Artificial Sequence
  Synthetic Construct
AEAEDVGVYYCMQQQEAPLTFGGGTK

SEQ ID NO: 101 - protein, 16 aa, Artificial Sequence
  Synthetic Construct
SGTASVVCLLNNFYPR

SEQ ID NO: 102 - protein, 20 aa, Artificial Sequence
  Synthetic Construct
VDNALQSGNSQESVTEQDSK

SEQ ID NO: 103 - protein, 330 aa, Artificial Sequence
  Synthetic Construct
ASTKGPSVFPLAPSSKSTSGGTAALGCLVKDYFPEPVTVSWNSGALTSGVHTFPAVLQSSGLYSLSSVVTVPSSSLGTQTYICNVNHKPSNTKVDKKVEPKSCDKTHTCPPCPAPEAAGGPSVFLFPPKPKDTLMISRTPEVTCVVVDVSHEDPEVKFNWYVDGVEVHNAKTKPREEQYNSTYRVVSVLTVLHQDWLNGKEYKCKVSNKALPASIEKTISKAKGQPREPQVYTLPPSRDELTKNQVSLTCLVKGFYPSDIAVEWESNGQPENNYKTTPPVLDSDGSFFLYSKLTVDKSRWQQGNVFSCSVMHEALHNHYTQKSLSLSPGK

SEQ ID NO: 104 - protein, 329 aa, Artificial Sequence
  Synthetic Construct
ASTKGPSVFPLAPSSKSTSGGTAALGCLVKDYFPEPVTVSWNSGALTSGVHTFPAVLQSSGLYSLSSVVTVPSSSLGTQTYICNVNHKPSNTKVDKKVEPKSCDKTHTCPPCPAPEAAGGPSVFLFPPKPKDTLMISRTPEVTCVVVDVSHEDPEVKFNWYVDGVEVHNAKTKPREEQYNSTYRVVSVLTVLHQDWLNGKEYKCKVSNKALPASIEKTISKAKGQPREPQVYTLPPSRDELTKNQVSLTCLVKGFYPSDIAVEWESNGQPENNYKTTPPVLDSDGSFFLYSKLTVDKSRWQQGNVFSCSVMHEALHNHYTQKSLSLSPG

SEQ ID NO: 105 - protein, 452 aa, Artificial Sequence
  Synthetic Construct
QVQLQESGPGLVKPSETLSLTCAVSGYSISSGYYWGWIRQPPGKGLEWIGTIYHSGSTYYNPSLKSQVTISVDTSKNQFSLELSSVTAADTAVYYCARQGSIQQGYYGMDVWGQGTTVTVSSASTKGPSVFPLAPSSKSTSGGTAALGCLVKDYFPEPVTVSWNSGALTSGVHTFPAVLQSSGLYSLSSVVTVPSSSLGTQTYICNVNHKPSNTKVDKKVEPKSCDKTHTCPPCPAPEAAGGPSVFLFPPKPKDTLMISRTPEVTCVVVDVSHEDPEVKFNWYVDGVEVHNAKTKPREEQYNSTYRVVSVLTVLHQDWLNGKEYKCKVSNKALPASIEKTISKAKGQPREPQVYTLPPSRDELTKNQVSLTCLVKGFYPSDIAVEWESNGQPENNYKTTPPVLDSDGSFFLYSKLTVDKSRWQQGNVFSCSVMHEALHNHYTQKSLSLSPGK

SEQ ID NO: 106 - protein, 451 aa, Artificial Sequence
  Synthetic Construct
QVQLQESGPGLVKPSETLSLTCAVSGYSISSGYYWGWIRQPPGKGLEWIGTIYHSGSTYYNPSLKSQVTISVDTSKNQFSLELSSVTAADTAVYYCARQGSIQQGYYGMDVWGQGTTVTVSSASTKGPSVFPLAPSSKSTSGGTAALGCLVKDYFPEPVTVSWNSGALTSGVHTFPAVLQSSGLYSLSSVVTVPSSSLGTQTYICNVNHKPSNTKVDKKVEPKSCDKTHTCPPCPAPEAAGGPSVFLFPPKPKDTLMISRTPEVTCVVVDVSHEDPEVKFNWYVDGVEVHNAKTKPREEQYNSTYRVVSVLTVLHQDWLNGKEYKCKVSNKALPASIEKTISKAKGQPREPQVYTLPPSRDELTKNQVSLTCLVKGFYPSDIAVEWESNGQPENNYKTTPPVLDSDGSFFLYSKLTVDKSRWQQGNVFSCSVMHEALHNHYTQKSLSLSPG

SEQ ID NO: 107 - protein, 122 aa, Artificial Sequence
  Synthetic Construct
QVQLQESGPGLVKPSETLSLTCAVSGYSISSVRYWGWIRQPPGKGLEWIGSIYHSGSTYYNPSLKSRVTISVDTSKNQFSLKLSSVTAADTAVYYCARQGSIKQGYYGMDVWGQGTTVTVSS

SEQ ID NO: 108 - protein, 122 aa, Artificial Sequence
  Synthetic Construct
QVQLQESGPGLVKPSETLSLTCAVSGYSISSVRYWGWIRQPPGKGLEWIGAIYPSGSTYYNPSLKSRVTISVDTSKNQFSLKLSSVTAADTAVYYCARQGSIKQGYYGMDVWGQGTTVTVSS

SEQ ID NO: 109 - protein, 122 aa, Artificial Sequence; identical to SEQ ID NO: 56
  Synthetic Construct

SEQ ID NO: 110 - protein, 122 aa, Artificial Sequence; identical to SEQ ID NO: 56
  Synthetic Construct

SEQ ID NO: 111 - protein, 122 aa, Artificial Sequence; identical to SEQ ID NO: 56
  Synthetic Construct

SEQ ID NO: 112 - protein, 122 aa, Artificial Sequence; identical to SEQ ID NO: 56
  Synthetic Construct

SEQ ID NO: 113 - protein, 112 aa, Artificial Sequence; identical to SEQ ID NO: 79
  Synthetic Construct

SEQ ID NO: 114 - protein, 112 aa, Artificial Sequence; identical to SEQ ID NO: 79
  Synthetic Construct

SEQ ID NO: 115 - protein, 112 aa, Artificial Sequence; identical to SEQ ID NO: 59
  Synthetic Construct

SEQ ID NO: 116 - protein, 112 aa, Artificial Sequence
  Synthetic Construct
DIVMTQSPLSLPVTPGESASISCRSSQGLLRSNGYNYLDWYLQKPGQSPQLLIYLGSNRASGVPDRFSGSGSGTDFTLKISRVEAEDVGVYYCMQQQETPLTFGGGTKVEIK

SEQ ID NO: 117 - protein, 112 aa, Artificial Sequence
  Synthetic Construct
DIVMTQSPLSLPVTPGEPASISCRSSQSLLRSNGYNYLDWYLQKPGQSPQLLIYLGSNRASGVPDRFSGSGSGTDFTLKISRVEAEDVGVYYCMQQQETPLTFGGGTKVEIK

SEQ ID NO: 118 - protein, 112 aa, Artificial Sequence
  Synthetic Construct
DIVMTQSPLSLPVTPGGPASISCRSSQSLLRSNGYNYLDWYLQKPGQSPQLLIYLGSNRASGVPDRFSGSGSGTDFTLKISRVEAEDVGVYYCMQQQETPLTFGGGTKVEIK

SEQ ID NO: 119 - protein, 219 aa, Artificial Sequence
  Synthetic Construct
DIVMTQSPLSLPVTPGEPASISCRSSQSLLRSHGYNYLDWYLQKPGQSPQLLIYLGSNRASGVPDRFSGSGSGTDFTLKISRAEAEDVGVYYCMQQQEAPLTFGGGTKVEIKRTVAAPSVFIFPPSDEQLKSGTASVVCLLNNFYPREAKVQWKVDNALQSGNSQESVTEQDSKDSTYSLSSTLTLSKADYEKHKVYACEVTHQGLSSPVTKSFNRGEC

SEQ ID NO: 120 - protein, 219 aa, Artificial Sequence
  Synthetic Construct
DIVMTQSPLSLPVTPGEPASISCRSSQSLLRSKGYNYLDWYLQKPGQSPQLLIYLGSNRASGVPDRFSGSGSGTDFTLKISRAEAEDVGVYYCMQQQEAPLTFGGGTKVEIKRTVAAPSVFIFPPSDEQLKSGTASVVCLLNNFYPREAKVQWKVDNALQSGNSQESVTEQDSKDSTYSLSSTLTLSKADYEKHKVYACEVTHQGLSSPVTKSFNRGEC

SEQ ID NO: 121 - protein, 219 aa, Artificial Sequence
  Synthetic Construct
DIVMTQSPLSLPVTPGEPASISCRSSQSLLRSQGYNYLDWYLQKPGQSPQLLIYLGSNRASGVPDRFSGSGSGTDFTLKISRAEAEDVGVYYCMQQQEAPLTFGGGTKVEIKRTVAAPSVFIFPPSDEQLKSGTASVVCLLNNFYPREAKVQWKVDNALQSGNSQESVTEQDSKDSTYSLSSTLTLSKADYEKHKVYACEVTHQGLSSPVTKSFNRGEC

SEQ ID NO: 122 - protein, 219 aa, Artificial Sequence
  Synthetic Construct
DIVMTQSPLSLPVTPGEPASISCRSSQSLLRSYGYNYLDWYLQKPGQSPQLLIYLGSNRASGVPDRFSGSGSGTDFTLKISRAEAEDVGVYYCMQQQEAPLTFGGGTKVEIKRTVAAPSVFIFPPSDEQLKSGTASVVCLLNNFYPREAKVQWKVDNALQSGNSQESVTEQDSKDSTYSLSSTLTLSKADYEKHKVYACEVTHQGLSSPVTKSFNRGEC

SEQ ID NO: 123 - protein, 219 aa, Artificial Sequence
  Synthetic Construct
DIVMTQSPLSLPVTPGEPASISCRSSQSLLRSEGYNYLDWYLQKPGQSPQLLIYLGSNRASGVPDRFSGSGSGTDFTLKISRAEAEDVGVYYCMQQQEAPLTFGGGTKVEIKRTVAAPSVFIFPPSDEQLKSGTASVVCLLNNFYPREAKVQWKVDNALQSGNSQESVTEQDSKDSTYSLSSTLTLSKADYEKHKVYACEVTHQGLSSPVTKSFNRGEC

SEQ ID NO: 124 - protein, 219 aa, Artificial Sequence
  Synthetic Construct
DIVMTQSPLSLPVTPGEPASISCRSSQSLLRSWGYNYLDWYLQKPGQSPQLLIYLGSNRASGVPDRFSGSGSGTDFTLKISRAEAEDVGVYYCMQQQEAPLTFGGGTKVEIKRTVAAPSVFIFPPSDEQLKSGTASVVCLLNNFYPREAKVQWKVDNALQSGNSQESVTEQDSKDSTYSLSSTLTLSKADYEKHKVYACEVTHQGLSSPVTKSFNRGEC

SEQ ID NO: 125 - protein, 219 aa, Artificial Sequence
  Synthetic Construct
DIVMTQSPLSLPVTPGEPASISCRSSQSLLRSFGYNYLDWYLQKPGQSPQLLIYLGSNRASGVPDRFSGSGSGTDFTLKISRAEAEDVGVYYCMQQQEAPLTFGGGTKVEIKRTVAAPSVFIFPPSDEQLKSGTASVVCLLNNFYPREAKVQWKVDNALQSGNSQESVTEQDSKDSTYSLSSTLTLSKADYEKHKVYACEVTHQGLSSPVTKSFNRGEC

SEQ ID NO: 126 - protein, 219 aa, Artificial Sequence
  Synthetic Construct
DIVMTQSPLSLPVTPGEPASISCRSSQSLLRSIGYNYLDWYLQKPGQSPQLLIYLGSNRASGVPDRFSGSGSGTDFTLKISRAEAEDVGVYYCMQQQEAPLTFGGGTKVEIKRTVAAPSVFIFPPSDEQLKSGTASVVCLLNNFYPREAKVQWKVDNALQSGNSQESVTEQDSKDSTYSLSSTLTLSKADYEKHKVYACEVTHQGLSSPVTKSFNRGEC

SEQ ID NO: 127 - protein, 219 aa, Artificial Sequence
  Synthetic Construct
DIVMTQSPLSLPVTPGEPASISCRSSQSLLRSVGYNYLDWYLQKPGQSPQLLIYLGSNRASGVPDRFSGSGSGTDFTLKISRAEAEDVGVYYCMQQQEAPLTFGGGTKVEIKRTVAAPSVFIFPPSDEQLKSGTASVVCLLNNFYPREAKVQWKVDNALQSGNSQESVTEQDSKDSTYSLSSTLTLSKADYEKHKVYACEVTHQGLSSPVTKSFNRGEC

SEQ ID NO: 128 - protein, 219 aa, Artificial Sequence
  Synthetic Construct
DIVMTQSPLSLPVTPGEPASISCRSSQSLLRSAGYNYLDWYLQKPGQSPQLLIYLGSNRASGVPDRFSGSGSGTDFTLKISRAEAEDVGVYYCMQQQEAPLTFGGGTKVEIKRTVAAPSVFIFPPSDEQLKSGTASVVCLLNNFYPREAKVQWKVDNALQSGNSQESVTEQDSKDSTYSLSSTLTLSKADYEKHKVYACEVTHQGLSSPVTKSFNRGEC

SEQ ID NO: 129 - protein, 219 aa, Artificial Sequence
  Synthetic Construct
DIVMTQSPLSLPVTPGEPASISCRSSQSLLRSMGYNYLDWYLQKPGQSPQLLIYLGSNRASGVPDRFSGSGSGTDFTLKISRAEAEDVGVYYCMQQQEAPLTFGGGTKVEIKRTVAAPSVFIFPPSDEQLKSGTASVVCLLNNFYPREAKVQWKVDNALQSGNSQESVTEQDSKDSTYSLSSTLTLSKADYEKHKVYACEVTHQGLSSPVTKSFNRGEC

SEQ ID NO: 130 - protein, 219 aa, Artificial Sequence
  Synthetic Construct
DIVMTQSPLSLPVTPGEPASISCRSSQSLLRSLGYNYLDWYLQKPGQSPQLLIYLGSNRASGVPDRFSGSGSGTDFTLKISRAEAEDVGVYYCMQQQEAPLTFGGGTKVEIKRTVAAPSVFIFPPSDEQLKSGTASVVCLLNNFYPREAKVQWKVDNALQSGNSQESVTEQDSKDSTYSLSSTLTLSKADYEKHKVYACEVTHQGLSSPVTKSFNRGEC

SEQ ID NO: 131 - protein, 219 aa, Artificial Sequence
  Synthetic Construct
DIVMTQSPLSLPVTPGEPASISCRSSQSLLRSNGYNYLDWYLQKPGQSPQLLIYLGSNRASGVPDRFSGSGSGTDFTLKISRVEAEDVGAYYCMQQQEAPLTFGGGTKVEIKRTVAAPSVFIFPPSDEQLKSGTASVVCLLNNFYPREAKVQWKVDNALQSGNSQESVTEQDSKDSTYSLSSTLTLSKADYEKHKVYACEVTHQGLSSPVTKSFNRGEC

SEQ ID NO: 132 - protein, 219 aa, Artificial Sequence
  Synthetic Construct
DIVMTQSPLSLPVTPGGPASISCRSSQSLLRSNGYNYLDWYLQKPGQSPQLLIYLGSNRASGVPDRLSGSGSGTDFTLKISRVEAEDVGVYYCMQQQETPLTFGGGTKVEIKRTVAAPSVFIFPPSDEQLKSGTASVVCLLNNFYPREAKVQWKVDNALQSGNSQESVTEQDSKDSTYSLSSTLTLSKADYEKHKVYACEVTHQGLSSPVTKSFNRGEC

SEQ ID NO: 133 - protein, 219 aa, Artificial Sequence
  Synthetic Construct
DIVMTQSPLSLPVTPGEPASISCRSSQSLLHSNGYNYLDWYLQKPGQSPQLLIYLGSNRASGVPDRFSGSGSGTDFTLKISRVEAEDVGVYYCMQQQETPLTFGGGTKVEIKRTVAAPSVFIFPPSDEQLKSGTASVVCLLNNFYPREAKVQWKVDNALQSGNSQESVTEQDSKDSTYSLSSTLTLSKADYEKHKVYACEVTHQGLSSPVTKSFNRGEC

SEQ ID NO: 134 - protein, 219 aa, Artificial Sequence
  Synthetic Construct
DIVMTQSPLSLPVTPGESASISCRSSQGLLRSNGYNYLDWYLQKPGQSPQLLIYLGSNRASGVPDRFSGSGSGTDFTLKISRVEAEDVGVYYCMQQQEAPLTFGGGTKVEIKRTVAAPSVFIFPPSDEQLKSGTASVVCLLNNFYPREAKVQWKVDNALQSGNSQESVTEQDSKDSTYSLSSTLTLSKADYEKHKVYACEVTHQGLSSPVTKSFNRGEC

SEQ ID NO: 135 - protein, 452 aa, Artificial Sequence
  Synthetic Construct
QVQLQESGPGLVKPSETLSLTCAVSGYSISSGYYWGWIRQPPGKGLEWIGTIYHSGSTYYNPSLESRVTISVDTSKNQFSLKLSSVTAADTAVYYCARQGSIQQGYYGMDVWGQGTTVTVSSASTKGPSVFPLAPSSKSTSGGTAALGCLVKDYFPEPVTVSWNSGALTSGVHTFPAVLQSSGLYSLSSVVTVPSSSLGTQTYICNVNHKPSNTKVDKKVEPKSCDKTHTCPPCPAPEAAGGPSVFLFPPKPKDTLMISRTPEVTCVVVDVSHEDPEVKFNWYVDGVEVHNAKTKPREEQYNSTYRVVSVLTVLHQDWLNGKEYKCKVSNKALPASIEKTISKAKGQPREPQVYTLPPSRDELTKNQVSLTCLVKGFYPSDIAVEWESNGQPENNYKTTPPVLDSDGSFFLYSKLTVDKSRWQQGNVFSCSVMHEALHNHYTQKSLSLSPGK

SEQ ID NO: 136 - protein, 451 aa, Artificial Sequence
  Synthetic Construct
QVQLQESGPGLVKPSETLSLTCAVSGYSISSGYYWGWIRQPPGKGLEWIGTIYHSGSTYYNPSLESRVTISVDTSKNQFSLKLSSVTAADTAVYYCARQGSIQQGYYGMDVWGQGTTVTVSSASTKGPSVFPLAPSSKSTSGGTAALGCLVKDYFPEPVTVSWNSGALTSGVHTFPAVLQSSGLYSLSSVVTVPSSSLGTQTYICNVNHKPSNTKVDKKVEPKSCDKTHTCPPCPAPEAAGGPSVFLFPPKPKDTLMISRTPEVTCVVVDVSHEDPEVKFNWYVDGVEVHNAKTKPREEQYNSTYRVVSVLTVLHQDWLNGKEYKCKVSNKALPASIEKTISKAKGQPREPQVYTLPPSRDELTKNQVSLTCLVKGFYPSDIAVEWESNGQPENNYKTTPPVLDSDGSFFLYSKLTVDKSRWQQGNVFSCSVMHEALHNHYTQKSLSLSPG

SEQ ID NO: 137 - protein, 452 aa, Artificial Sequence
  Synthetic Construct
QVQLQESGPGLVKPSETLSLTCAVSGYSISSGYYWGWIRQPPGKGLEWIGTIYHSGSTYYNPSLKSRVTISVDTSKNQFSLKLSSVTAADTAVYYCARQGSIKQGYYGMDVWGQGTTVTVSSASTKGPSVFPLAPSSKSTSGGTAALGCLVKDYFPEPVTVSWNSGALTSGVHTFPAVLQSSGLYSLSSVVTVPSSSLGTQTYICNVNHKPSNTKVDKKVEPKSCDKTHTCPPCPAPEAAGGPSVFLFPPKPKDTLMISRTPEVTCVVVDVSHEDPEVKFNWYVDGVEVHNAKTKPREEQYNSTYRVVSVLTVLHQDWLNGKEYKCKVSNKALPASIEKTISKAKGQPREPQVYTLPPSRDELTKNQVSLTCLVKGFYPSDIAVEWESNGQPENNYKTTPPVLDSDGSFFLYSKLTVDKSRWQQGNVFSCSVMHEALHNHYTQKSLSLSPGK

SEQ ID NO: 138 - protein, 451 aa, Artificial Sequence
  Synthetic Construct
QVQLQESGPGLVKPSETLSLTCAVSGYSISSGYYWGWIRQPPGKGLEWIGTIYHSGSTYYNPSLKSRVTISVDTSKNQFSLKLSSVTAADTAVYYCARQGSIKQGYYGMDVWGQGTTVTVSSASTKGPSVFPLAPSSKSTSGGTAALGCLVKDYFPEPVTVSWNSGALTSGVHTFPAVLQSSGLYSLSSVVTVPSSSLGTQTYICNVNHKPSNTKVDKKVEPKSCDKTHTCPPCPAPEAAGGPSVFLFPPKPKDTLMISRTPEVTCVVVDVSHEDPEVKFNWYVDGVEVHNAKTKPREEQYNSTYRVVSVLTVLHQDWLNGKEYKCKVSNKALPASIEKTISKAKGQPREPQVYTLPPSRDELTKNQVSLTCLVKGFYPSDIAVEWESNGQPENNYKTTPPVLDSDGSFFLYSKLTVDKSRWQQGNVFSCSVMHEALHNHYTQKSLSLSPG

SEQ ID NO: 139 - protein, 219 aa, Artificial Sequence
  Synthetic Construct
DIVMTQSPLSLPVTPGEPASISCRSSQSLLRSNGYNYLDWYLQKPGQSPQLLIYLGSNRASGVPDRFSGSGSGTDFTLKISRAEAEDVGVYYCMQQQEAPLTFGGGTKVEIKRTVAAPSVFIFPPSDEQLKSGTASVVCLLNNFYPREAKVQWKVDNALQSGNSQESVTEQDSKDSTYSLSSTLTLSKADYEKHKVYACEVTHQGLSSPVTKSFNRGEC

SEQ ID NO: 140 - protein, 219 aa, Artificial Sequence
  Synthetic Construct
DIVMTQSPLSLPVTPGEPASISCRSSQSLLRSNGYNYLDWYLQKPGQSPQLLIYLGSNRASGVPDRFSGSGSGTDFTLKISRVEAEDVGVYYCMQQQEAPLTFGGGTKVEIKRTVAAPSVFIFPPSDEQLKSGTASVVCLLNNFYPREAKVQWKVDNALQSGNSQESVTEQDSKDSTYSLSSTLTLSKADYEKHKVYACEVTHQGLSSPVTKSFNRGEC

SEQ ID NO: 141 - protein, 219 aa, Artificial Sequence
  Synthetic Construct
DIVMTQSPLSLPVTPGEPASISCRSSQSLLRSNGYNYLDWYLQKPGQPPQLLIYLGSNRVSGVPDRFSGSGSGTDFTLKISRVEAEDVGVYYCMQQQETPLTFGGGTKVEIKRTVAAPSVFIFPPSDEQLKSGTASVVCLLNNFYPREAKVQWKVDNALQSGNSQESVTEQDSKDSTYSLSSTLTLSKADYEKHKVYACEVTHQGLSSPVTKSFNRGEC

SEQ ID NO: 142 - protein, 219 aa, Artificial Sequence
  Synthetic Construct
DIVMTQSPLSLPVTPGEPASISCRSSQSLLRSTGYNYLDWYLQKPGQSPQLLIYLGSNRASGVPDRFSGSGSGTDFTLKISRAEAEDVGVYYCMQQQEAPLTFGGGTKVEIKRTVAAPSVFIFPPSDEQLKSGTASVVCLLNNFYPREAKVQWKVDNALQSGNSQESVTEQDSKDSTYSLSSTLTLSKADYEKHKVYACEVTHQGLSSPVTKSFNRGEC

SEQ ID NO: 143 - protein, 219 aa, Artificial Sequence
  Synthetic Construct
DIVMTQSPLSLPVTPGEPASISCRSSQSLLRSSGYNYLDWYLQKPGQSPQLLIYLGSNRASGVPDRFSGSGSGTDFTLKISRAEAEDVGVYYCMQQQEAPLTFGGGTKVEIKRTVAAPSVFIFPPSDEQLKSGTASVVCLLNNFYPREAKVQWKVDNALQSGNSQESVTEQDSKDSTYSLSSTLTLSKADYEKHKVYACEVTHQGLSSPVTKSFNRGEC

SEQ ID NO: 144 - protein, 219 aa, Artificial Sequence
  Synthetic Construct
DIVMTQSPLSLPVTPGEPASISCRSSQSLLRSGGYNYLDWYLQKPGQSPQLLIYLGSNRASGVPDRFSGSGSGTDFTLKISRAEAEDVGVYYCMQQQEAPLTFGGGTKVEIKRTVAAPSVFIFPPSDEQLKSGTASVVCLLNNFYPREAKVQWKVDNALQSGNSQESVTEQDSKDSTYSLSSTLTLSKADYEKHKVYACEVTHQGLSSPVTKSFNRGEC

SEQ ID NO: 145 - protein, 219 aa, Artificial Sequence
  Synthetic Construct
DIVMTQSPLSLPVTPGEPASISCRSSQSLLRSRGYNYLDWYLQKPGQSPQLLIYLGSNRASGVPDRFSGSGSGTDFTLKISRAEAEDVGVYYCMQQQEAPLTFGGGTKVEIKRTVAAPSVFIFPPSDEQLKSGTASVVCLLNNFYPREAKVQWKVDNALQSGNSQESVTEQDSKDSTYSLSSTLTLSKADYEKHKVYACEVTHQGLSSPVTKSFNRGEC

SEQ ID NO: 146 - protein, 219 aa, Artificial Sequence
  Synthetic Construct
DIVMTQSPLSLPVTPGEPASISCRSSQSLLRSDGYNYLDWYLQKPGQSPQLLIYLGSNRASGVPDRFSGSGSGTDFTLKISRAEAEDVGVYYCMQQQEAPLTFGGGTKVEIKRTVAAPSVFIFPPSDEQLKSGTASVVCLLNNFYPREAKVQWKVDNALQSGNSQESVTEQDSKDSTYSLSSTLTLSKADYEKHKVYACEVTHQGLSSPVTKSFNRGEC